European Patent Specification EP 3 979 790 B1, published April 15, 2026. Title: NON-HUMAN ANIMALS HAVING A LIMITED LAMBDA LIGHT CHAIN REPERTOIRE EXPRESSED FROM THE KAPPA LOCUS AND USES THEREOF. Applicant: REGENERON PHARMACEUTICALS, INC. The sequence listing filed with the application follows.

SEQUENCE LISTING (73 sequences)

SEQ ID NO: 1 - DNA, 317 bp, Mus sp.
gccagcccaagtcttcgccatcagtcaccctgtttccaccttcctctgaagagctcgagactaacaaggccacactggtgtgtacgatcactgatttctacccaggtgtggtgacagtggactggaaggtagatggtacccctgtcactcagggtatggagacaacccagccttccaaacagagcaacaacaagtacatggctagcagctacctgaccctgacagcaagagcatgggaaaggcatagcagttacagctgccaggtcactcatgaaggtcacactgtggagaagagtttgtcccgtgctgactgttcc

SEQ ID NO: 2 - DNA, 314 bp, Mus sp.
gtcagcccaagtccactcccactctcaccgtgtttccaccttcctctgaggagctcaaggaaaacaaagccacactggtgtgtctgatttccaacttttccccgagtggtgtgacagtggcctggaaggcaaatggtacacctatcacccagggtgtggacacttcaaatcccaccaaagagggcaacaagttcatggccagcagcttcctacatttgacatcggaccagtggagatctcacaacagttttacctgtcaagttacacatgaaggggacactgtggagaagagtctgtctcctgcagaatgtctc

SEQ ID NO: 3 - DNA, 314 bp, Mus sp.
gtcagcccaagtccactcccacactcaccatgtttccaccttcccctgaggagctccaggaaaacaaagccacactcgtgtgtctgatttccaatttttccccaagtggtgtgacagtggcctggaaggcaaatggtacacctatcacccagggtgtggacacttcaaatcccaccaaagaggacaacaagtacatggccagcagcttcttacatttgacatcggaccagtggagatctcacaacagttttacctgccaagttacacatgaaggggacactgtggagaagagtctgtctcctgcagaatgtctc

SEQ ID NO: 4 - protein, 106 aa, Mus sp.
GQPKSSPSVTLFPPSSEELETNKATLVCTITDFYPGVVTVDWKVDGTPVTQGMETTQPSKQSNNKYMASSYLTLTARAWERHSSYSCQVTHEGHTVEKSLSRADCS

SEQ ID NO: 5 - protein, 105 aa, Mus sp.
GQPKSTPTLTVFPPSSEELKENKATLVCLISNFSPSGVTVAWKANGTPITQGVDTSNPTKEGNKFMASSFLHLTSDQWRSHNSFTCQVTHEGDTVEKSLSPAECL

SEQ ID NO: 6 - protein, 105 aa, Mus sp.
GQPKSTPTLTMFPPSPEELQENKATLVCLISNFSPSGVTVAWKANGTPITQGVDTSNPTKEDNKYMASSFLHLTSDQWRSHNSFTCQVTHEGDTVEKSLSPAECL

SEQ ID NO: 7 - DNA, 314 bp, Rattus sp.
gtcagcccaagtccactcccacactcacagtatttccaccttcaactgaggagctccagggaaacaaagccacactggtgtgtctgatttctgatttctacccgagtgatgtggaagtggcctggaaggcaaatggtgcacctatctcccagggtgtggacactgcaaatcccaccaaacagggcaacaaatacatcgccagcagcttcttacgtttgacagcagaacagtggagatctcgcaacagttttacctgccaagttacacatgaagggaacactgtggagaagagtctgtctcctgcagaatgtgtc

SEQ ID NO: 8 - DNA, 314 bp, Rattus sp.
accaacccaaggctacgccctcagtcaccctgttcccaccttcctctgaagagctcaagactgacaaggctacactggtgtgtatggtgacagatttctaccctggtgttatgacagtggtctggaaggcagatggtacccctatcactcagggtgtggagactacccagcctttcaaacagaacaacaagtacatggctaccagctacctgcttttgacagcaaaagcatgggagactcatagcaattacagctgccaggtcactcacgaagagaacactgtggagaagagtttgtcccgtgctgagtgttcc

SEQ ID NO: 9 - DNA, 314 bp, Rattus sp.
gtcagcccaagtccactcccacactcacagtatttccaccttcaactgaggagctccagggaaacaaagccacactggtgtgtctgatttctgatttctacccgagtgatgtggaagtggcctggaaggcaaatggtgcacctatctcccagggtgtggacactgcaaatcccaccaaacagggcaacaaatacatcgccagcagcttcttacgtttgacagcagaacagtggagatctcgcaacagttttacctgccaagttacacatgaagggaacactgtggaaaagagtctgtctcctgcagagtgtgtc

SEQ ID NO: 10 - DNA, 314 bp, Rattus sp.; identical to SEQ ID NO: 8

SEQ ID NO: 11 - protein, 105 aa, Rattus sp.
GQPKSTPTLTVFPPSTEELQGNKATLVCLISDFYPSDVEVAWKANGAPISQGVDTANPTKQGNKYIASSFLRLTAEQWRSRNSFTCQVTHEGNTVEKSLSPAECV

SEQ ID NO: 12 - protein, 105 aa, Rattus sp.
DQPKATPSVTLFPPSSEELKTDKATLVCMVTDFYPGVMTVVWKADGTPITQGVETTQPFKQNNKYMATSYLLLTAKAWETHSNYSCQVTHEENTVEKSLSRAECS

SEQ ID NO: 13 - protein, 105 aa, Rattus sp.; identical to SEQ ID NO: 11

SEQ ID NO: 14 - protein, 105 aa, Rattus sp.; identical to SEQ ID NO: 12

SEQ ID NO: 15 - DNA, 315 bp, Homo sapiens
cccaaggccaaccccacggtcactctgttcccgccctcctctgaggagctccaagccaacaaggccacactagtgtgtctgatcagtgacttctacccgggagctgtgacagtggcttggaaggcagatggcagccccgtcaaggcgggagtggagacgaccaaaccctccaaacagagcaacaacaagtacgcggccagcagctacctgagcctgacgcccgagcagtggaagtcccacagaagctacagctgccaggtcacgcatgaagggagcaccgtggagaagacagtggcccctacagaatgttcatag

SEQ ID NO: 16 - DNA, 317 bp, Homo sapiens
gtcagcccaaggctgccccctcggtcactctgttcccgccctcctctgaggagcttcaagccaacaaggccacactggtgtgtctcataagtgacttctacccgggagccgtgacagtggcttggaaagcagatagcagccccgtcaaggcgggagtggagaccaccacaccctccaaacaaagcaacaacaagtacgcggccagcagctatctgagcctgacgcctgagcagtggaagtcccacagaagctacagctgccaggtcacgcatgaagggagcaccgtggagaagacagtggcccctacagaatgttca

SEQ ID NO: 17 - DNA, 315 bp, Homo sapiens
cccaaggctgccccctcggtcactctgttcccaccctcctctgaggagcttcaagccaacaaggccacactggtgtgtctcataagtgacttctacccgggagccgtgacagttgcctggaaggcagatagcagccccgtcaaggcgggggtggagaccaccacaccctccaaacaaagcaacaacaagtacgcggccagcagctacctgagcctgacgcctgagcagtggaagtcccacaaaagctacagctgccaggtcacgcatgaagggagcaccgtggagaagacagttgcccctacggaatgttcatag

SEQ ID NO: 18 - DNA, 321 bp, Homo sapiens
ggtcagcccaaggctgccccatcggtcactctgttcccgccctcctctgaggagcttcaagccaacaaggccacactggtgtgcctgatcagtgacttctacccgggagctgtgaaagtggcctggaaggcagatggcagccccgtcaacacgggagtggagaccaccacaccctccaaacagagcaacaacaagtacgcggccagcagctacctgagcctgacgcctgagcagtggaagtcccacagaagctacagctgccaggtcacgcatgaagggagcaccgtggagaagacagtggcccctgcagaatgttcatag

SEQ ID NO: 19 - DNA, 317 bp, Homo sapiens
gtcagcccaaggctgccccctcggtcactctgttcccaccctcctctgaggagcttcaagccaacaaggccacactggtgtgtctcgtaagtgacttctacccgggagccgtgacagtggcctggaaggcagatggcagccccgtcaaggtgggagtggagaccaccaaaccctccaaacaaagcaacaacaagtatgcggccagcagctacctgagcctgacgcccgagcagtggaagtcccacagaagctacagctgccgggtcacgcatgaagggagcaccgtggagaagacagtggcccctgcagaatgctct

SEQ ID NO: 20 - protein, 104 aa, Homo sapiens
PKANPTVTLFPPSSEELQANKATLVCLISDFYPGAVTVAWKADGSPVKAGVETTKPSKQSNNKYAASSYLSLTPEQWKSHRSYSCQVTHEGSTVEKTVAPTECS

SEQ ID NO: 21 - protein, 105 aa, Homo sapiens
QPKAAPSVTLFPPSSEELQANKATLVCLISDFYPGAVTVAWKADSSPVKAGVETTTPSKQSNNKYAASSYLSLTPEQWKSHRSYSCQVTHEGSTVEKTVAPTECS

SEQ ID NO: 22 - protein, 104 aa, Homo sapiens
PKAAPSVTLFPPSSEELQANKATLVCLISDFYPGAVTVAWKADSSPVKAGVETTTPSKQSNNKYAASSYLSLTPEQWKSHKSYSCQVTHEGSTVEKTVAPTECS

SEQ ID NO: 23 - protein, 105 aa, Homo sapiens
QPKAAPSVTLFPPSSEELQANKATLVCLISDFYPGAVKVAWKADGSPVNTGVETTTPSKQSNNKYAASSYLSLTPEQWKSHRSYSCQVTHEGSTVEKTVAPAECS

SEQ ID NO: 24 - protein, 105 aa, Homo sapiens
QPKAAPSVTLFPPSSEELQANKATLVCLVSDFYPGAVTVAWKADGSPVKVGVETTKPSKQSNNKYAASSYLSLTPEQWKSHRSYSCRVTHEGSTVEKTVAPAECS

SEQ ID NO: 25 - DNA, 532 bp, Mus sp.
gggctgatgctgcaccaactgtatccatcttcccaccatccagtgagcagttaacatctggaggtgcctcagtcgtgtgcttcttgaacaacttctaccccaaagacatcaatgtcaagtggaagattgatggcagtgaacgacaaaatggcgtcctgaacagttggactgatcaggacagcaaagacagcacctacagcatgagcagcaccctcacgttgaccaaggacgagtatgaacgacataacagctatacctgtgaggccactcacaagacatcaacttcacccattgtcaagagcttcaacaggaatgagtgttagagacaaaggtcctgagacgccaccaccagctccccagctccatcctatcttcccttctaaggtcttggaggcttccccacaagcgacctaccactgttgcggtgctccaaacctcctccccacctccttctcctcctcctccctttccttggcttttatcatgctaatatttgcagaaaatattcaataaagtgagtctttgcacttga

SEQ ID NO: 26 - protein, 106 aa, Mus sp.
ADAAPTVSIFPPSSEQLTSGGASVVCFLNNFYPKDINVKWKIDGSERQNGVLNSWTDQDSKDSTYSMSSTLTLTKDEYERHNSYTCEATHKTSTSPIVKSFNRNEC

SEQ ID NO: 27 - DNA, 521 bp, Rattus sp.
gggctgatgctgcaccaactgtatctatcttcccaccatccacggaacagttagcaactggaggtgcctcagtcgtgtgcctcatgaacaacttctatcccagagacatcagtgtcaagtggaagattgatggcactgaacgacgagatggtgtcctggacagtgttactgatcaggacagcaaagacagcacgtacagcatgagcagcaccctctcgttgaccaaggctgactatgaaagtcataacctctatacctgtgaggttgttcataagacatcatcctcacccgtcgtcaagagcttcaacaggaatgagtgttagacccaaaggtcctgaggtgccacctgctccccagctccttccaatcttccctcctaaggtcttggagacttccccacaagcgacctaccactgttgcggtgctccaaacctcctccccacctcatcctccttcctttccttggctttgatcatgctaatatttggggaatattaaataaagtgaatctttgcacttga

SEQ ID NO: 28 - protein, 106 aa, Rattus sp.
ADAAPTVSIFPPSTEQLATGGASVVCLMNNFYPRDISVKWKIDGTERRDGVLDSVTDQDSKDSTYSMSSTLSLTKADYESHNLYTCEVVHKTSSSPVVKSFNRNEC

SEQ ID NO: 29 - DNA, 320 bp, Homo sapiens
gaactgtggctgcaccatctgtcttcatcttcccgccatctgatgagcagttgaaatctggaactgcctctgttgtgtgcctgctgaataacttctatcccagagaggccaaagtacagtggaaggtggataacgccctccaatcgggtaactcccaggagagtgtcacagagcaggacagcaaggacagcacctacagcctcagcagcaccctgacgctgagcaaagcagactacgagaaacacaaagtctacgcctgcgaagtcacccatcagggcctgagctcgcccgtcacaaagagcttcaacaggggagagtgt

SEQ ID NO: 30 - protein, 106 aa, Homo sapiens
TVAAPSVFIFPPSDEQLKSGTASVVCLLNNFYPREAKVQWKVDNALQSGNSQESVTEQDSKDSTYSLSSTLTLSKADYEKHKVYACEVTHQGLSSPVTKSFNRGEC

SEQ ID NO: 31 - DNA, 2992 bp, Artificial Sequence
  source: /note="Description of Artificial Sequence: Synthetic polynucleotide"
ggcgcgccacctgcagtgtacacctgaggtgacatggttctgaacatcactttccccattgaaggcccgagtgacctatcacttgcttctcaaaattcaggaactaggtgactctaggagagtgcacaggaagctttctgcatattctttcaagagatttcgaggtcactgactcttttttcaagacttaaacacaaaatccacatccatcattcttgcgtaaagagaccattcttttttttttgagatggagtctcgctctgttgcccaagctggagtgcagtggcatgatctcggctcactgcaagctctgtcttctgggttcatgcccttctcctgcctcagcctcccaagtagctgggactacaggcacccgccgccatgcccggctaattttttgtattttttagtggagatggggtttcaacatgttggccagaatggtcttgatctcttgacctcgtgatccacccgccttggcctcccaaagtgctgggattacaggtgtgagccactgcacccggcccaagatggggtttcatcatgttgacctggctggtctcaaactcccaacctcaagtgatccactcacttcagcctcccaaagtgctgggatgacaggcgtgagccacagtgcccggcctagtacattgtttaaatggtgcatgtaaaacctcatggtactacaactgcctggtgacagactcaccagagtaaataactatcctgctgttctccaaccacatgggattccccaaacaaagatttgttgagtccaagatgcatcatgccagaactcttgcagtcatacacataatttgtttcattttaataaatacggttatcttttttcttcagtttattgtttttaatgtatcatcttctaggtttcattacacatcaaagatgaataatttctctcatctttaggacatgctgaaaacactcattagtgattttgaacagtattatttcctaaacatcctagttggaatggttgatcctaaaagctaccatgtgtcaggctcacctgagtgcagactgtggtctaaacaagctaaagttttaattcttccatcttcaaatacggagcatatttgcttgttttgctctttagcaaaacactgcaaagtcattcgccaggatctcctgcagactggcattcagtgatggagaacagactcctaggtgagatccctggtcacaggatccagatgactatgactgcaagtctggaaaagaagagacagaacaaagatttaccagcataaccctctgagaatgtgccccagccatcctggagggaagagctccctattgacccagcactgcagaatccacagaggaaggacagctctggccaccagggagcagccacacgacaagagaggacccggtgtccccacaggtgaggaaatgagtccatggggctggtcagtgctctcgatttcattctgccataacaggactttgtgtagtcaccacctgagtcctatacagtgaacagccaaggagacatggacagattcacccctgaggaacccagtagaatgtgaagtctgccctgaggtcacgaagaaaagactcggggggctgcctggcctggccctgatggagggggccatggacagaacaacggggaggcaggggtgtctctgagaggctctggtcaccttgtcatacaatggtggtgtacaatgtcgcaccatggacactagggggcgcctgcgcaccattcctgagaagactgggtgtgatgagagcaggaccagcgccacctgtcctgcttggtgccctatgcttagggctcacagatgtcaactctccaccccctgggaccacacagccccacccctggcactctctgacatcctcaggcagaggagcttgacccagggcccagggtgggatcagaaagctggagggtctgatttgcatggatggaccctccttctctcagagtataaagaggggcagggagagacttggggaagctctgcttcagctgtgagcgcagaaggcaggactcgggacaatcttcatcatgacctgctcccctctcctcctcacccttctcattcactgcacaggtgcccagacacagggtcaggggaggggtccaggaagcccatgaggccctgctttctccttctctctctagaccaagaatcaccgtgtctgtgtctctcctgcttccagggtcctgggcccagtctgtgttgacgcagccgccctcagtgtctgcggccccaggacagaaggtcaccatctcctgctctggaagcagctccaacattgggaataattatgtatcctggtaccagcagctcccaggaacagcccccaaactcctcatttatgacaataataagcgaccctcagggattcctgaccgattctctggctccaagtctggcacgtcagccaccctgggcatcaccggactccagactggggacgaggccgattattactgcggaacatgggatagcagcctgagtgctgtggtattcggcggagggaccaagctgaccgtcctaggtaagtaatttttcactattgtcttctgaaatttgggtctgatggccagtattgacttttagaggcttaaataggagtttggtaaagattggtaaatgagggcatttaagatttgccatgggttgcaaaagttaaactcagcttcaaaaatggatttggagaaaaaaagattaaattgctctaaactgaatgacacaaagtaaaaaaaaaaagtgtaactaaaaaggaacccttgtatttctaaggagcaaaagtaaatttatttttgttcactcttgccaaatattgtattggttgttgctgattatgcatgatacagaaaagtggaaaaatacattttttagtctttctcccttttgtttgataaattattttgtcagacaacaataaaaatcaatagcacgccctaagatgccatttcattacctctttctccgcacccgacatagat

SEQ ID NO: 32 - DNA, 497 bp, Artificial Sequence
  source: /note="Description of Artificial Sequence: Synthetic polynucleotide"
atgacctgctcccctctcctcctcacccttctcattcactgcacaggtgcccagacacagggtcaggggaggggtccaggaagcccatgaggccctgctttctccttctctctctagaccaagaatcaccgtgtctgtgtctctcctgcttccagggtcctgggcccagtctgtgttgacgcagccgccctcagtgtctgcggccccaggacagaaggtcaccatctcctgctctggaagcagctccaacattgggaataattatgtatcctggtaccagcagctcccaggaacagcccccaaactcctcatttatgacaataataagcgaccctcagggattcctgaccgattctctggctccaagtctggcacgtcagccaccctgggcatcaccggactccagactggggacgaggccgattattactgcggaacatgggatagcagcctgagtgctgtggtattcggcggagggaccaagctgaccgtcctag

SEQ ID NO: 33 - DNA, 388 bp, Artificial Sequence
  source: /note="Description of Artificial Sequence: Synthetic polynucleotide"
atgacctgctcccctctcctcctcacccttctcattcactgcacagggtcctgggcccagtctgtgttgacgcagccgccctcagtgtctgcggccccaggacagaaggtcaccatctcctgctctggaagcagctccaacattgggaataattatgtatcctggtaccagcagctcccaggaacagcccccaaactcctcatttatgacaataataagcgaccctcagggattcctgaccgattctctggctccaagtctggcacgtcagccaccctgggcatcaccggactccagactggggacgaggccgattattactgcggaacatgggatagcagcctgagtgctgtggtattcggcggagggaccaagctgaccgtcctag

SEQ ID NO: 34 - protein, 129 aa, Artificial Sequence
  source: /note="Description of Artificial Sequence: Synthetic polypeptide"
MTCSPLLLTLLIHCTGSWAQSVLTQPPSVSAAPGQKVTISCSGSSSNIGNNYVSWYQQLPGTAPKLLIYDNNKRPSGIPDRFSGSKSGTSATLGITGLQTGDEADYYCGTWDSSLSAVVFGGGTKLTVL

SEQ ID NO: 35 - protein, 110 aa, Artificial Sequence
  source: /note="Description of Artificial Sequence: Synthetic polypeptide"
QSVLTQPPSVSAAPGQKVTISCSGSSSNIGNNYVSWYQQLPGTAPKLLIYDNNKRPSGIPDRFSGSKSGTSATLGITGLQTGDEADYYCGTWDSSLSAVVFGGGTKLTVL

SEQ ID NO: 36 - DNA, 3003 bp, Artificial Sequence
  source: /note="Description of Artificial Sequence: Synthetic polynucleotide"
ggcgcgccacctgcagtgtacacctgaggtgacatggttctgaacatcactttccccattgaaggcccgagtgacctatcacttgcttctcaaaattcaggaactaggtgactctaggagagtgcacaggaagctttctgcatattctttcaagagatttcgaggtcactgactcttttttcaagacttaaacacaaaatccacatccatcattcttgcgtaaagagaccattcttttttttttgagatggagtctcgctctgttgcccaagctggagtgcagtggcatgatctcggctcactgcaagctctgtcttctgggttcatgcccttctcctgcctcagcctcccaagtagctgggactacaggcacccgccgccatgcccggctaattttttgtattttttagtggagatggggtttcaacatgttggccagaatggtcttgatctcttgacctcgtgatccacccgccttggcctcccaaagtgctgggattacaggtgtgagccactgcacccggcccaagatggggtttcatcatgttgacctggctggtctcaaactcccaacctcaagtgatccactcacttcagcctcccaaagtgctgggatgacaggcgtgagccacagtgcccggcctagtacattgtttaaatggtgcatgtaaaacctcatggtactacaactgcctggtgacagactcaccagagtaaataactatcctgctgttctccaaccacatgggattccccaaacaaagatttgttgagtccaagatgcatcatgccagaactcttgcagtcatacacataatttgtttcattttaataaatacggttatcttttttcttcagtttattgtttttaatgtatcatcttctaggtttcattacacatcaaagatgaataatttctctcatctttaggacatgctgaaaacactcattagtgattttgaacagtattatttcctaaacatcctagttggaatggttgatcctaaaagctaccatgtgtcaggctcacctgagtgcagactgtggtctaaacaagctaaagttttaattcttccatcttcaaatacggagcatatttgcttgttttgctctttagcaaaacactgcaaagtcattcgccaggatctcctgcagactggcattcagtgatggagaacagactcctaggtgagatccctggtcacaggatccagatgactatgactgcaagtctggaaaagaagagacagaacaaagatttaccagcataaccctctgagaatgtgccccagccatcctggagggaagagctccctattgacccagcactgcagaatccacagaggaaggacagctctggccaccagggagcagccacacgacaagagaggacccggtgtccccacaggtgaggaaatgagtccatggggctggtcagtgctctcgatttcattctgccataacaggactttgtgtagtcaccacctgagtcctatacagtgaacagccaaggagacatggacagattcacccctgaggaacccagtagaatgtgaagtctgccctgaggtcacgaagaaaagactcggggggctgcctggcctggccctgatggagggggccatggacagaacaacggggaggcaggggtgtctctgagaggctctggtcaccttgtcatacaatggtggtgtacaatgtcgcaccatggacactagggggcgcctgcgcaccattcctgagaagactgggtgtgatgagagcaggaccagcgccacctgtcctgcttggtgccctatgcttagggctcacagatgtcaactctccaccccctgggaccacacagccccacccctggcactctctgacatcctcaggcagaggagcttgacccagggcccagggtgggatcagaaagctggagggtctgatttgcatggatggaccctccttctctcagagtataaagaggggcagggagagacttggggaagctctgcttcagctgtgagcgcagaaggcaggactcgggacaatcttcatcatggcctgggctctgctgctcctcaccctcctcactcagggcacaggtgacgcctccagggaaggggcttcagggacctctgggctgatccttggtctcctgctcctcaggctcaccggggcccagcactgactcactggcatgtgtttctccctctttccagggtcctgggcccagtctgccctgactcagcctgcctccgtgtctgggtctcctggacagtcgatcaccatctcctgcactggaaccagcagtgacgttggtggttataactatgtctcctggtaccaacagcacccaggcaaagcccccaaactcatgatttatgaggtcagtaatcggccctcaggggtttctaatcgcttctctggctccaagtctggcaacacggcctccctgaccatctctgggctccaggctgaggacgaggctgattattactgcagctcatatacaagcagcagcactctcgtggtattcggcggagggaccaagctgaccgtcctaggtaagtaatttttcactattgtcttctgaaatttgggtctgatggccagtattgacttttagaggcttaaataggagtttggtaaagattggtaaatgagggcatttaagatttgccatgggttgcaaaagttaaactcagcttcaaaaatggatttggagaaaaaaagattaaattgctctaaactgaatgacacaaagtaaaaaaaaaaagtgtaactaaaaaggaacccttgtatttctaaggagcaaaagtaaatttatttttgttcactcttgccaaatattgtattggttgttgctgattatgcatgatacagaaaagtggaaaaatacattttttagtctttctcccttttgtttgataaattattttgtcagacaacaataaaaatcaatagcacgccctaagatgccatttcattacctctttctccgcacccgacatagat

SEQ ID NO: 37 - DNA, 508 bp, Artificial Sequence
  source: /note="Description of Artificial Sequence: Synthetic polynucleotide"
atggcctgggctctgctgctcctcaccctcctcactcagggcacaggtgacgcctccagggaaggggcttcagggacctctgggctgatccttggtctcctgctcctcaggctcaccggggcccagcactgactcactggcatgtgtttctccctctttccagggtcctgggcccagtctgccctgactcagcctgcctccgtgtctgggtctcctggacagtcgatcaccatctcctgcactggaaccagcagtgacgttggtggttataactatgtctcctggtaccaacagcacccaggcaaagcccccaaactcatgatttatgaggtcagtaatcggccctcaggggtttctaatcgcttctctggctccaagtctggcaacacggcctccctgaccatctctgggctccaggctgaggacgaggctgattattactgcagctcatatacaagcagcagcactctcgtggtattcggcggagggaccaagctgaccgtcctag

SEQ ID NO: 38 - DNA, 391 bp, Artificial Sequence
  source: /note="Description of Artificial Sequence: Synthetic polynucleotide"
atggcctgggctctgctgctcctcaccctcctcactcagggcacagggtcctgggcccagtctgccctgactcagcctgcctccgtgtctgggtctcctggacagtcgatcaccatctcctgcactggaaccagcagtgacgttggtggttataactatgtctcctggtaccaacagcacccaggcaaagcccccaaactcatgatttatgaggtcagtaatcggccctcaggggtttctaatcgcttctctggctccaagtctggcaacacggcctccctgaccatctctgggctccaggctgaggacgaggctgattattactgcagctcatatacaagcagcagcactctcgtggtattcggcggagggaccaagctgaccgtcctag

SEQ ID NO: 39 - protein, 130 aa, Artificial Sequence
  source: /note="Description of Artificial Sequence: Synthetic polypeptide"
MAWALLLLTLLTQGTGSWAQSALTQPASVSGSPGQSITISCTGTSSDVGGYNYVSWYQQHPGKAPKLMIYEVSNRPSGVSNRFSGSKSGNTASLTISGLQAEDEADYYCSSYTSSSTLVVFGGGTKLTVL

SEQ ID NO: 40 - protein, 111 aa, Artificial Sequence
  source: /note="Description of Artificial Sequence: Synthetic polypeptide"
QSALTQPASVSGSPGQSITISCTGTSSDVGGYNYVSWYQQHPGKAPKLMIYEVSNRPSGVSNRFSGSKSGNTASLTISGLQAEDEADYYCSSYTSSSTLVVFGGGTKLTVL

SEQ ID NO: 41 - DNA, 22 bp, Artificial Sequence
  source: /note="Description of Artificial Sequence: Synthetic primer"
gggacgaggccgattattactg

SEQ ID NO: 42 - DNA, 23 bp, Artificial Sequence
  source: /note="Description of Artificial Sequence: Synthetic probe"
cggaacatgggatagcagcctga

SEQ ID NO: 43 - DNA, 18 bp, Artificial Sequence
  source: /note="Description of Artificial Sequence: Synthetic primer"
cctccgccgaataccaca

SEQ ID NO: 44 - DNA, 20 bp, Artificial Sequence
  source: /note="Description of Artificial Sequence: Synthetic primer"
gcatcaccggactccagact

SEQ ID NO: 45 - DNA, 25 bp, Artificial Sequence
  source: /note="Description of Artificial Sequence: Synthetic probe"
cgaggccgattattactgcggaaca

SEQ ID NO: 46 - DNA, 18 bp, Artificial Sequence
  source: /note="Description of Artificial Sequence: Synthetic primer"
aggacggtcagcttggtc

SEQ ID NO: 47 - DNA, 23 bp, Artificial Sequence
  source: /note="Description of Artificial Sequence: Synthetic primer"
caggactcgggacaatcttcatc

SEQ ID NO: 48 - DNA, 21 bp, Artificial Sequence
  source: /note="Description of Artificial Sequence: Synthetic probe"
atggcctgggctctgctgctc

SEQ ID NO: 49 - DNA, 18 bp, Artificial Sequence
  source: /note="Description of Artificial Sequence: Synthetic primer"
tgtgccctgagtgaggag

SEQ ID NO: 50 - DNA, 19 bp, Artificial Sequence
  source: /note="Description of Artificial Sequence: Synthetic primer"
agcgcagaaggcaggactc

SEQ ID NO: 51 - DNA, 25 bp, Artificial Sequence
  source: /note="Description of Artificial Sequence: Synthetic probe"
acaatcttcatcatggcctgggctc

SEQ ID NO: 52 - DNA, 18 bp, Artificial Sequence
  source: /note="Description of Artificial Sequence: Synthetic primer"
cgtcacctgtgccctgag

SEQ ID NO: 53 - DNA, 19 bp, Artificial Sequence
  source: /note="Description of Artificial Sequence: Synthetic primer"
tgttgcccaagctggagtg

SEQ ID NO: 54 - DNA, 22 bp, Artificial Sequence
  source: /note="Description of Artificial Sequence: Synthetic probe"
tggcatgatctcggctcactgc

SEQ ID NO: 55 - DNA, 18 bp, Artificial Sequence
  source: /note="Description of Artificial Sequence: Synthetic primer"
gaggctgaggcaggagaa

SEQ ID NO: 56 - DNA, 21 bp, Artificial Sequence
  source: /note="Description of Artificial Sequence: Synthetic primer"
ggccactcacaagacatcaac

SEQ ID NO: 57 - DNA, 25 bp, Artificial Sequence
  source: /note="Description of Artificial Sequence: Synthetic probe"
tcacccattgtcaagagcttcaaca

SEQ ID NO: 58 - DNA, 24 bp, Artificial Sequence
  source: /note="Description of Artificial Sequence: Synthetic primer"
cgtctcaggacctttgtctctaac

SEQ ID NO: 59 - DNA, 25 bp, Artificial Sequence
  source: /note="Description of Artificial Sequence: Synthetic primer"
tccttgttacttcataccatcctct

SEQ ID NO: 60 - DNA, 20 bp, Artificial Sequence
  source: /note="Description of Artificial Sequence: Synthetic probe"
ttccttcctcaggccagccc

SEQ ID NO: 61 - DNA, 22 bp, Artificial Sequence
  source: /note="Description of Artificial Sequence: Synthetic primer"
agggtgactgatggcgaagact

SEQ ID NO: 62 - DNA, 19 bp, Artificial Sequence
  source: /note="Description of Artificial Sequence: Synthetic primer"
tccaggcaccctgtctttg

SEQ ID NO: 63 - DNA, 24 bp, Artificial Sequence
  source: /note="Description of Artificial Sequence: Synthetic probe"
aaagagccaccctctcctgcaggg

SEQ ID NO: 64 - DNA, 26 bp, Artificial Sequence
  source: /note="Description of Artificial Sequence: Synthetic primer"
aagtagctgctgctaacactctgact

SEQ ID NO: 65 - DNA, 28 bp, Artificial Sequence
  source: /note="Description of Artificial Sequence: Synthetic primer"
aggtgagggtacagataagtgttatgag

SEQ ID NO: 66 - DNA, 29 bp, Artificial Sequence
  source: /note="Description of Artificial Sequence: Synthetic probe"
ccattatgatgctccatgcctctctgttc

SEQ ID NO: 67 - DNA, 27 bp, Artificial Sequence
  source: /note="Description of Artificial Sequence: Synthetic primer"
tgacaaatgccctaattatagtgatca

SEQ ID NO: 68 - DNA, 19 bp, Artificial Sequence
  source: /note="Description of Artificial Sequence: Synthetic primer"
ggtggagaggctattcggc

SEQ ID NO: 69 - DNA, 23 bp, Artificial Sequence
  source: /note="Description of Artificial Sequence: Synthetic probe"
tgggcacaacagacaatcggctg

SEQ ID NO: 70 - DNA, 17 bp, Artificial Sequence
  source: /note="Description of Artificial Sequence: Synthetic primer"
gaacacggcggcatcag

SEQ ID NO: 71 - DNA, 17 bp, Artificial Sequence
  source: /note="Description of Artificial Sequence: Synthetic primer"
tgcggccgatcttagcc

SEQ ID NO: 72 - DNA, 21 bp, Artificial Sequence
  source: /note="Description of Artificial Sequence: Synthetic probe"
acgagcgggttcggcccattc

SEQ ID NO: 73 - DNA, 18 bp, Artificial Sequence
  source: /note="Description of Artificial Sequence: Synthetic primer"
ttgaccgattccttgcgg